European Patent Specification EP 3 887 403 B1, published July 15, 2026. Title: ANTI-4-1BB ANTIBODY AND USE THEREOF. Applicant: ABL Bio Inc. The sequence listing filed with the application follows.

SEQUENCE LISTING (67 sequences)

SEQ ID NO: 1 - protein, 5 aa, Artificial Sequence
  Synthetic_CDR-H1 of anti-4-1BB antibody
SYDMS

SEQ ID NO: 2 - protein, 5 aa, Artificial Sequence
  Synthetic_CDR-H1 of anti-4-1BB antibody
GYDMS

SEQ ID NO: 3 - protein, 5 aa, Artificial Sequence
  Synthetic_CDR-H1 of anti-4-1BB antibody
SNVMN

SEQ ID NO: 4 - protein, 17 aa, Artificial Sequence
  Synthetic_CDR-H2 of anti-4-1BB antibody
WISYSGGSIYYADSVKG

SEQ ID NO: 5 - protein, 17 aa, Artificial Sequence
  Synthetic_CDR-H2 of anti-4-1BB antibody
VIYPDDGNTYYADSVKG

SEQ ID NO: 6 - protein, 16 aa, Artificial Sequence
  Synthetic_CDR-H2 of anti-4-1BB antibody
EISHSGSTNYNPSLKS

SEQ ID NO: 7 - protein, 12 aa, Artificial Sequence
  Synthetic_CDR-H3 of anti-4-1BB antibody
DGQRNSMREFDY

SEQ ID NO: 8 - protein, 12 aa, Artificial Sequence
  Synthetic_CDR-H3 of anti-4-1BB antibody
DAQRNSMREFDY

SEQ ID NO: 9 - protein, 12 aa, Artificial Sequence
  Synthetic_CDR-H3 of anti-4-1BB antibody
DAQRQSMREFDY

SEQ ID NO: 10 - protein, 18 aa, Artificial Sequence
  Synthetic_CDR-H3 of anti-4-1BB antibody
HGGQKPTTKSSSAYGMDG

SEQ ID NO: 11 - protein, 7 aa, Artificial Sequence
  Synthetic_CDR-H3 of anti-4-1BB antibody
GAGNLGY

SEQ ID NO: 12 - protein, 13 aa, Artificial Sequence
  Synthetic_CDR-L1 of anti-4-1BB antibody
SGSSSNIGNNYVT

SEQ ID NO: 13 - protein, 11 aa, Artificial Sequence
  Synthetic_CDR-L1 of anti-4-1BB antibody
QASQDISNYLN

SEQ ID NO: 14 - protein, 7 aa, Artificial Sequence
  Synthetic_CDR-L2 of anti-4-1BB antibody
ADSHRPS

SEQ ID NO: 15 - protein, 7 aa, Artificial Sequence
  Synthetic_CDR-L2 of anti-4-1BB antibody
GASSRAT

SEQ ID NO: 16 - protein, 11 aa, Artificial Sequence
  Synthetic_CDR-L3 of anti-4-1BB antibody
ATWDYSLSGYV

SEQ ID NO: 17 - protein, 9 aa, Artificial Sequence
  Synthetic_CDR-L3 of anti-4-1BB antibody
QQYNSYPIT

SEQ ID NO: 18 - protein, 121 aa, Artificial Sequence
  Synthetic_Heavy chain variable region of anti-4-1BB antibody
EVQLLESGGGLVQPGGSLRLSCAASGFTFSSYDMSWVRQAPGKGLEWVSWISYSGGSIYYADSVKGRFTISRDNSKNTLYLQMNSLRAEDTAVYYCARDGQRNSMREFDYWGQGTLVTVSS

SEQ ID NO: 19 - protein, 121 aa, Artificial Sequence
  Synthetic_Heavy chain variable region of anti-4-1BB antibody
EVQLLESGGGLVQPGGSLRLSCAASGFTFSSYDMSWVRQAPGKGLEWVSWISYSGGSIYYADSVKGRFTISRDNSKNTLYLQMNSLRAEDTAVYYCARDAQRNSMREFDYWGQGTLVTVSS

SEQ ID NO: 20 - protein, 121 aa, Artificial Sequence
  Synthetic_Heavy chain variable region of anti-4-1BB antibody
EVQLLESGGGLVQPGGSLRLSCAASGFTFSSYDMSWVRQAPGKGLEWVSWISYSGGSIYYADSVKGRFTISRDNSKNTLYLQMNSLRAEDTAVYYCARDAQRQSMREFDYWGQGTLVTVSS

SEQ ID NO: 21 - protein, 127 aa, Artificial Sequence
  Synthetic_Heavy chain variable region of anti-4-1BB antibody
EVQLLESGGGLVQPGGSLRLSCAASGFTFSGYDMSWVRQAPGKGLEWVSVIYPDDGNTYYADSVKGRFTISRDNSKNTLYLQMNSLRAEDAAVYYCAKHGGQKPTTKSSSAYGMDGWGQGTLVTVSS

SEQ ID NO: 22 - protein, 127 aa, Artificial Sequence
  Synthetic_Heavy chain variable region of anti-4-1BB antibody
EVQLLESGGGLVQPGGSLRLSCAASGFTFSGYDMSWVRQAPGKGLEWVSVIYPDDGNTYYADSVKGRFTISRDNSKNTLYLQMNSLRAEDTAVYYCAKHGGQKPTTKSSSAYGMDGWGQGTLVTVSS

SEQ ID NO: 23 - protein, 115 aa, Artificial Sequence
  Synthetic_Heavy chain variable region of anti-4-1BB antibody
EVQLLESGGGLVQPGGSLRLSCAASGFTFSSNVMNWVRQAPGKGLEWVSEISHSGSTNYNPSLKSRFTISRDNSKNTLYLQMNSLRAEDTAVYYCAVGAGNLGYWGQGTLVTVSS

SEQ ID NO: 24 - protein, 110 aa, Artificial Sequence
  Synthetic_Light chain variable region of anti-4-1BB antibody
QSVLTQPPSASGTPGRRVTISCSGSSSNIGNNYVTWYQQLPGTAPKLLIYADSHRPSGVPDRFSGSKSGTSASLAISGLRSEDEADYYCATWDYSLSGYVFGGGTKLTVL

SEQ ID NO: 25 - protein, 110 aa, Artificial Sequence
  Synthetic_Light chain variable region of anti-4-1BB antibody
QSVLTQPPSASGTPGQRVTISCSGSSSNIGNNYVTWYQQLPGTAPKLLIYADSHRPSGVPDRFSGSKSGTSASLAISGLRSEDEADYYCATWDYSLSGYVFGGGTKLTVL

SEQ ID NO: 26 - protein, 108 aa, Artificial Sequence
  Synthetic_Light chain variable region of anti-4-1BB antibody
EIVLTQSPGTLSLSPGERATLSCQASQDISNYLNWYQQKPGQAPRLLIYGASSRATGIPDRFSGSGSGTDFTLTISRLEPEDFAVYYCQQYNSYPITFGQGTKLEIKR

SEQ ID NO: 27 - protein, 448 aa, Artificial Sequence
  Synthetic_Heavy chain of anti-4-1BB antibody
EVQLLESGGGLVQPGGSLRLSCAASGFTFSSYDMSWVRQAPGKGLEWVSWISYSGGSIYYADSVKGRFTISRDNSKNTLYLQMNSLRAEDTAVYYCARDGQRNSMREFDYWGQGTLVTVSSASTKGPSVFPLAPCSRSTSESTAALGCLVKDYFPEPVTVSWNSGALTSGVHTFPAVLQSSGLYSLSSVVTVPSSSLGTKTYTCNVDHKPSNTKVDKRVESKYGPPCPPCPAPEFLGGPSVFLFPPKPKDTLMISRTPEVTCVVVDVSQEDPEVQFNWYVDGVEVHNAKTKPREEQFNSTYRVVSVLTVLHQDWLNGKEYKCKVSNKGLPSSIEKTISKAKGQPREPQVYTLPPSQEEMTKNQVSLTCLVKGFYPSDIAVEWESNGQPENNYKTTPPVLDSDGSFFLYSRLTVDKSRWQEGNVFSCSVMHEALHNHYTQKSLSLSLGK

SEQ ID NO: 28 - protein, 448 aa, Artificial Sequence
  Synthetic_Heavy chain of anti-4-1BB antibody
EVQLLESGGGLVQPGGSLRLSCAASGFTFSSYDMSWVRQAPGKGLEWVSWISYSGGSIYYADSVKGRFTISRDNSKNTLYLQMNSLRAEDTAVYYCARDAQRNSMREFDYWGQGTLVTVSSASTKGPSVFPLAPCSRSTSESTAALGCLVKDYFPEPVTVSWNSGALTSGVHTFPAVLQSSGLYSLSSVVTVPSSSLGTKTYTCNVDHKPSNTKVDKRVESKYGPPCPPCPAPEFLGGPSVFLFPPKPKDTLMISRTPEVTCVVVDVSQEDPEVQFNWYVDGVEVHNAKTKPREEQFNSTYRVVSVLTVLHQDWLNGKEYKCKVSNKGLPSSIEKTISKAKGQPREPQVYTLPPSQEEMTKNQVSLTCLVKGFYPSDIAVEWESNGQPENNYKTTPPVLDSDGSFFLYSRLTVDKSRWQEGNVFSCSVMHEALHNHYTQKSLSLSLGK

SEQ ID NO: 29 - protein, 448 aa, Artificial Sequence
  Synthetic_Heavy chain of anti-4-1BB antibody
EVQLLESGGGLVQPGGSLRLSCAASGFTFSSYDMSWVRQAPGKGLEWVSWISYSGGSIYYADSVKGRFTISRDNSKNTLYLQMNSLRAEDTAVYYCARDAQRQSMREFDYWGQGTLVTVSSASTKGPSVFPLAPCSRSTSESTAALGCLVKDYFPEPVTVSWNSGALTSGVHTFPAVLQSSGLYSLSSVVTVPSSSLGTKTYTCNVDHKPSNTKVDKRVESKYGPPCPPCPAPEFLGGPSVFLFPPKPKDTLMISRTPEVTCVVVDVSQEDPEVQFNWYVDGVEVHNAKTKPREEQFNSTYRVVSVLTVLHQDWLNGKEYKCKVSNKGLPSSIEKTISKAKGQPREPQVYTLPPSQEEMTKNQVSLTCLVKGFYPSDIAVEWESNGQPENNYKTTPPVLDSDGSFFLYSRLTVDKSRWQEGNVFSCSVMHEALHNHYTQKSLSLSLGK

SEQ ID NO: 30 - protein, 454 aa, Artificial Sequence
  Synthetic_Heavy chain of anti-4-1BB antibody
EVQLLESGGGLVQPGGSLRLSCAASGFTFSGYDMSWVRQAPGKGLEWVSVIYPDDGNTYYADSVKGRFTISRDNSKNTLYLQMNSLRAEDAAVYYCAKHGGQKPTTKSSSAYGMDGWGQGTLVTVSSASTKGPSVFPLAPCSRSTSESTAALGCLVKDYFPEPVTVSWNSGALTSGVHTFPAVLQSSGLYSLSSVVTVPSSSLGTKTYTCNVDHKPSNTKVDKRVESKYGPPCPPCPAPEFLGGPSVFLFPPKPKDTLMISRTPEVTCVVVDVSQEDPEVQFNWYVDGVEVHNAKTKPREEQFNSTYRVVSVLTVLHQDWLNGKEYKCKVSNKGLPSSIEKTISKAKGQPREPQVYTLPPSQEEMTKNQVSLTCLVKGFYPSDIAVEWESNGQPENNYKTTPPVLDSDGSFFLYSRLTVDKSRWQEGNVFSCSVMHEALHNHYTQKSLSLSLGK

SEQ ID NO: 31 - protein, 454 aa, Artificial Sequence
  Synthetic_Heavy chain of anti-4-1BB antibody
EVQLLESGGGLVQPGGSLRLSCAASGFTFSGYDMSWVRQAPGKGLEWVSVIYPDDGNTYYADSVKGRFTISRDNSKNTLYLQMNSLRAEDTAVYYCAKHGGQKPTTKSSSAYGMDGWGQGTLVTVSSASTKGPSVFPLAPCSRSTSESTAALGCLVKDYFPEPVTVSWNSGALTSGVHTFPAVLQSSGLYSLSSVVTVPSSSLGTKTYTCNVDHKPSNTKVDKRVESKYGPPCPPCPAPEFLGGPSVFLFPPKPKDTLMISRTPEVTCVVVDVSQEDPEVQFNWYVDGVEVHNAKTKPREEQFNSTYRVVSVLTVLHQDWLNGKEYKCKVSNKGLPSSIEKTISKAKGQPREPQVYTLPPSQEEMTKNQVSLTCLVKGFYPSDIAVEWESNGQPENNYKTTPPVLDSDGSFFLYSRLTVDKSRWQEGNVFSCSVMHEALHNHYTQKSLSLSLGK

SEQ ID NO: 32 - protein, 442 aa, Artificial Sequence
  Synthetic_Heavy chain of anti-4-1BB antibody
EVQLLESGGGLVQPGGSLRLSCAASGFTFSSNVMNWVRQAPGKGLEWVSEISHSGSTNYNPSLKSRFTISRDNSKNTLYLQMNSLRAEDTAVYYCAVGAGNLGYWGQGTLVTVSSASTKGPSVFPLAPCSRSTSESTAALGCLVKDYFPEPVTVSWNSGALTSGVHTFPAVLQSSGLYSLSSVVTVPSSSLGTKTYTCNVDHKPSNTKVDKRVESKYGPPCPPCPAPEFLGGPSVFLFPPKPKDTLMISRTPEVTCVVVDVSQEDPEVQFNWYVDGVEVHNAKTKPREEQFNSTYRVVSVLTVLHQDWLNGKEYKCKVSNKGLPSSIEKTISKAKGQPREPQVYTLPPSQEEMTKNQVSLTCLVKGFYPSDIAVEWESNGQPENNYKTTPPVLDSDGSFFLYSRLTVDKSRWQEGNVFSCSVMHEALHNHYTQKSLSLSLGK

SEQ ID NO: 33 - protein, 216 aa, Artificial Sequence
  Synthetic_Light chain of anti-4-1BB antibody
QSVLTQPPSASGTPGRRVTISCSGSSSNIGNNYVTWYQQLPGTAPKLLIYADSHRPSGVPDRFSGSKSGTSASLAISGLRSEDEADYYCATWDYSLSGYVFGGGTKLTVLGQPKAAPSVTLFPPSSEELQANKATLVCLISDFYPGAVTVAWKADSSPVKAGVETTTPSKQSNNKYAASSYLSLTPEQWKSHRSYSCQVTHEGSTVEKTVAPAECS

SEQ ID NO: 34 - protein, 216 aa, Artificial Sequence
  Synthetic_Light chain of anti-4-1BB antibody
QSVLTQPPSASGTPGQRVTISCSGSSSNIGNNYVTWYQQLPGTAPKLLIYADSHRPSGVPDRFSGSKSGTSASLAISGLRSEDEADYYCATWDYSLSGYVFGGGTKLTVLGQPKAAPSVTLFPPSSEELQANKATLVCLISDFYPGAVTVAWKADSSPVKAGVETTTPSKQSNNKYAASSYLSLTPEQWKSHRSYSCQVTHEGSTVEKTVAPAECS

SEQ ID NO: 35 - protein, 108 aa, Artificial Sequence; identical to SEQ ID NO: 26
  Synthetic_Light chain of anti-4-1BB antibody

SEQ ID NO: 36 - protein, 327 aa, Artificial Sequence
  Synthetic_Heavy chain constant region
ASTKGPSVFPLAPCSRSTSESTAALGCLVKDYFPEPVTVSWNSGALTSGVHTFPAVLQSSGLYSLSSVVTVPSSSLGTKTYTCNVDHKPSNTKVDKRVESKYGPPCPPCPAPEFLGGPSVFLFPPKPKDTLMISRTPEVTCVVVDVSQEDPEVQFNWYVDGVEVHNAKTKPREEQFNSTYRVVSVLTVLHQDWLNGKEYKCKVSNKGLPSSIEKTISKAKGQPREPQVYTLPPSQEEMTKNQVSLTCLVKGFYPSDIAVEWESNGQPENNYKTTPPVLDSDGSFFLYSRLTVDKSRWQEGNVFSCSVMHEALHNHYTQKSLSLSLGK

SEQ ID NO: 37 - protein, 106 aa, Artificial Sequence
  Synthetic_Light chain constant region
GQPKAAPSVTLFPPSSEELQANKATLVCLISDFYPGAVTVAWKADSSPVKAGVETTTPSKQSNNKYAASSYLSLTPEQWKSHRSYSCQVTHEGSTVEKTVAPAECS

SEQ ID NO: 38 - protein, 106 aa, Artificial Sequence
  Synthetic_Light chain constant region
TVAAPSVFIFPPSDEQLKSGTASVVCLLNNFYPREAKVQWKVDNALQSGNSQESVTEQDSKDSTYSLSSTLTLSKADYEKHKVYACEVTHQGLSSPVTKSFNRGEC

SEQ ID NO: 39 - protein, 121 aa, Artificial Sequence
  Synthetic_Heavy chain variable region of anti-4-1BB scFv
EVQLLESGGGLVQPGGSLRLSCAASGFTFSSYDMSWVRQAPGKCLEWVSWISYSGGSIYYADSVKGRFTISRDNSKNTLYLQMNSLRAEDTAVYYCARDAQRQSMREFDYWGQGTLVTVSS

SEQ ID NO: 40 - protein, 30 aa, Artificial Sequence
  Synthetic_H-FR1 of anti-4-1BB antibody
EVQLLESGGGLVQPGGSLRLSCAASGFTFS

SEQ ID NO: 41 - protein, 14 aa, Artificial Sequence
  Synthetic_H-FR2 of anti-4-1BB antibody
WVRQAPGKGLEWVS

SEQ ID NO: 42 - protein, 32 aa, Artificial Sequence
  Synthetic_H-FR3 of anti-4-1BB antibody
RFTISRDNSKNTLYLQMNSLRAEDTAVYYCAR

SEQ ID NO: 43 - protein, 32 aa, Artificial Sequence
  Synthetic_H-FR3 of anti-4-1BB antibody
RFTISRDNSKNTLYLQMNSLRAEDAAVYYCAK

SEQ ID NO: 44 - protein, 32 aa, Artificial Sequence
  Synthetic_H-FR3 of anti-4-1BB antibody
RFTISRDNSKNTLYLQMNSLRAEDTAVYYCAK

SEQ ID NO: 45 - protein, 32 aa, Artificial Sequence
  Synthetic_H-FR3 of anti-4-1BB antibody
RFTISRDNSKNTLYLQMNSLRAEDTAVYYCAV

SEQ ID NO: 46 - protein, 11 aa, Artificial Sequence
  Synthetic_H-FR4 of anti-4-1BB antibody
WGQGTLVTVSS

SEQ ID NO: 47 - protein, 22 aa, Artificial Sequence
  Synthetic_L-FR1 of anti-4-1BB antibody
QSVLTQPPSASGTPGRRVTISC

SEQ ID NO: 48 - protein, 22 aa, Artificial Sequence
  Synthetic_L-FR1 of anti-4-1BB antibody
QSVLTQPPSASGTPGQRVTISC

SEQ ID NO: 49 - protein, 23 aa, Artificial Sequence
  Synthetic_L-FR1 of anti-4-1BB antibody
EIVLTQSPGTLSLSPGERATLSC

SEQ ID NO: 50 - protein, 15 aa, Artificial Sequence
  Synthetic_L-FR2 of anti-4-1BB antibody
WYQQLPGTAPKLLIY

SEQ ID NO: 51 - protein, 15 aa, Artificial Sequence
  Synthetic_L-FR2 of anti-4-1BB antibody
WYQQKPGQAPRLLIY

SEQ ID NO: 52 - protein, 32 aa, Artificial Sequence
  Synthetic_L-FR3 of anti-4-1BB antibody
GVPDRFSGSKSGTSASLAISGLRSEDEADYYC

SEQ ID NO: 53 - protein, 32 aa, Artificial Sequence
  Synthetic_L-FR3 of anti-4-1BB antibody
GIPDRFSGSGSGTDFTLTISRLEPEDFAVYYC

SEQ ID NO: 54 - protein, 10 aa, Artificial Sequence
  Synthetic_L-FR4 of anti-4-1BB antibody
FGGGTKLTVL

SEQ ID NO: 55 - protein, 11 aa, Artificial Sequence
  Synthetic_L-FR4 of anti-4-1BB antibody
FGQGTKLEIKR

SEQ ID NO: 56 - protein, 20 aa, Artificial Sequence
  Synthetic_Peptide linker
GGGGSGGGGSGGGGSGGGGS

SEQ ID NO: 57 - protein, 121 aa, Artificial Sequence
  Synthetic_Heavy chain variable region of anti-4-1BB scFv
EVQLLESGGGLVQPGGSLRLSCAASGFTFSSYDMSWVRQAPGKCLEWVSWISYSGGSIYYADSVKGRFTISRDNSKNTLYLQMNSLRAEDTAVYYCARDGQRNSMREFDYWGQGTLVTVSS

SEQ ID NO: 58 - protein, 121 aa, Artificial Sequence
  Synthetic_Heavy chain variable region of anti-4-1BB scFv
EVQLLESGGGLVQPGGSLRLSCAASGFTFSSYDMSWVRQAPGKCLEWVSWISYSGGSIYYADSVKGRFTISRDNSKNTLYLQMNSLRAEDTAVYYCARDAQRNSMREFDYWGQGTLVTVSS

SEQ ID NO: 59 - protein, 127 aa, Artificial Sequence
  Synthetic_Heavy chain variable region of anti-4-1BB scFv
EVQLLESGGGLVQPGGSLRLSCAASGFTFSGYDMSWVRQAPGKCLEWVSVIYPDDGNTYYADSVKGRFTISRDNSKNTLYLQMNSLRAEDAAVYYCAKHGGQKPTTKSSSAYGMDGWGQGTLVTVSS

SEQ ID NO: 60 - protein, 127 aa, Artificial Sequence
  Synthetic_Heavy chain variable region of anti-4-1BB scFv
EVQLLESGGGLVQPGGSLRLSCAASGFTFSGYDMSWVRQAPGKCLEWVSVIYPDDGNTYYADSVKGRFTISRDNSKNTLYLQMNSLRAEDTAVYYCAKHGGQKPTTKSSSAYGMDGWGQGTLVTVSS

SEQ ID NO: 61 - protein, 110 aa, Artificial Sequence
  Synthetic_Light chain variable region of anti-4-1BB scFv
QSVLTQPPSASGTPGRRVTISCSGSSSNIGNNYVTWYQQLPGTAPKLLIYADSHRPSGVPDRFSGSKSGTSASLAISGLRSEDEADYYCATWDYSLSGYVFGCGTKLTVL

SEQ ID NO: 62 - protein, 110 aa, Artificial Sequence
  Synthetic_Light chain variable region of anti-4-1BB scFv
QSVLTQPPSASGTPGQRVTISCSGSSSNIGNNYVTWYQQLPGTAPKLLIYADSHRPSGVPDRFSGSKSGTSASLAISGLRSEDEADYYCATWDYSLSGYVFGCGTKLTVL

SEQ ID NO: 63 - protein, 449 aa, Artificial Sequence
  Synthetic_Heavy Chain of anti-PD-L1 antibody
EVQLVESGGGLVQPGGSLRLSCAASGFTFSSYDMSWVRQAPGKSLEWVATISDAGGYIYYRDSVKGRFTISRDNAKNSLYLQMNSLRDEDTAVYICARELPWRYALDYWGQGTTVTVSSASTKGPSVFPLAPSSKSTSGGTAALGCLVKDYFPEPVTVSWNSGALTSGVHTFPAVLQSSGLYSLSSVVTVPSSSLGTQTYICNVNHKPSNTKVDKKVEPKSCDKTHTCPPCPAPELLGGPSVFLFPPKPKDTLMISRTPEVTCVVVDVSHEDPEVKFNWYVDGVEVHNAKTKPREEQYASTYRVVSVLTVLHQDWLNGKEYKCKVSNKALPAPIEKTISKAKGQPREPQVYTLPPSREEMTKNQVSLTCLVKGFYPSDIAVEWESNGQPENNYKTTPPVLDSDGSFFLYSKLTVDKSRWQQGNVFSCSVMHEALHNHYTQKSLSLSPGK

SEQ ID NO: 64 - protein, 214 aa, Artificial Sequence
  Synthetic_Light Chain of anti-PD-L1 antibody
DIQMTQSPSSLSASVGDRVTITCKASQDVTPAVAWYQQKPGKAPKLLIYSTSSRYTGVPSRFSGSGSGTDFTFTISSLQPEDIATYYCQQHYTTPLTFGQGTKLEIKRTVAAPSVFIFPPSDEQLKSGTASVVCLLNNFYPREAKVQWKVDNALQSGNSQESVTEQDSKDSTYSLSSTLTLSKADYEKHKVYACEVTHQGLSSPVTKSFNRGEC

SEQ ID NO: 65 - protein, 449 aa, Artificial Sequence
  Synthetic_Heavy Chain of anti-PD-L1 antibody
EVQLVESGGGLVQPGGSLRLSCAASGFTFSSYDMSWVRQAPGKSLEWVATISDAGGYIYYSDSVKGRFTISRDNAKNSLYLQMNSLRDEDTAVYICAREFGKRYALDYWGQGTTVTVSSASTKGPSVFPLAPSSKSTSGGTAALGCLVKDYFPEPVTVSWNSGALTSGVHTFPAVLQSSGLYSLSSVVTVPSSSLGTQTYICNVNHKPSNTKVDKKVEPKSCDKTHTCPPCPAPELLGGPSVFLFPPKPKDTLMISRTPEVTCVVVDVSHEDPEVKFNWYVDGVEVHNAKTKPREEQYASTYRVVSVLTVLHQDWLNGKEYKCKVSNKALPAPIEKTISKAKGQPREPQVYTLPPSREEMTKNQVSLTCLVKGFYPSDIAVEWESNGQPENNYKTTPPVLDSDGSFFLYSKLTVDKSRWQQGNVFSCSVMHEALHNHYTQKSLSLSPGK

SEQ ID NO: 66 - protein, 15 aa, Artificial Sequence
  Synthetic_Peptide linker
GGGGSGGGGSGGGGS

SEQ ID NO: 67 - protein, 255 aa, Artificial Sequence
  Synthetic_4-1BB protein (NP_001552.2)
MGNSCYNIVATLLLVLNFERTRSLQDPCSNCPAGTFCDNNRNQICSPCPPNSFSSAGGQRTCDICRQCKGVFRTRKECSSTSNAECDCTPGFHCLGAGCSMCEQDCKQGQELTKKGCKDCCFGTFNDQKRGICRPWTNCSLDGKSVLVNGTKERDVVCGPSPADLSPGASSVTPPAPAREPGHSPQIISFFLALTSTALLFLLFFLTLRFSVVKRGRKKLLYIFKQPFMRPVQTTQEEDGCSCRFPEEEEGGCEL